European Patent Application EP 4 714 974 A1, published March 25, 2026. Title: 双特异性抗原结合分子及其应用. Applicant: 上海齐鲁制药研究中心有限公司. Application WO. The sequence listing filed with the application follows.

SEQUENCE LISTING (28 sequences)

SEQ ID NO: 1 - protein, 707 aa, synthetic construct
QVQLVQSGAEVKKPGASVKVSCKASGYTFTSYIIHWVRQAPGQGLEWIGYINPYNDGTKYNEKFKGRVTMTSDTSTSTVYMELSSLRSEDTAVYYCARGGIRAFMNYWGQGTLVTVSSASTKGPSVFPLAPSSKSTSGGTAALGCLVKDYFPEPVTVSWNSGALTSGVHTFPAVLQSSGLYSLSSVVTVPSSSLGTQTYICNVNHKPSNTKVDKKVEPKSCGGGGSEVKLVESGGGLVQPGGSLKLSCAASGFTFNTYAMNWVRQAPGKGLEWVARIRSKYNNYATYYADSVKDRFTISRDDAKNTLYLQMNNLRTEDTAVYYCVRHGNFGNSYVSWFAYWGQGTLVTVSSGGGGSGGGGSGGGGSQAVVTQEPSLTVSPGGTVTLTCRSSTGAVTTSNYANWVQQKPGQAPRGLIGGTNKRAPGTPARFSGSLLGGKAALTLSGAQPEDEAEYYCALWYSNLWVFGGGTKLTVLEPKSSDKTHTCPPCPAPEAAGGPSVFLFPPKPKDTLMISRTPEVTCVVVDVSHEDPEVKFNWYVDGVEVHNAKTKPREEQYNSTYRVVSVLTVLHQDWLNGKEYKCKVSNKALPAPIEKTISKAKGQPREPQVYTLPPCRDELTKNQVSLWCLVKGFYPSDIAVEWESNGQPENNYKTTPPVLDSDGSFFLYSKLTVDKSRWQQGNVFSCSVMHEALHNHYTQKSLSLSPGK

SEQ ID NO: 2 - protein, 448 aa, synthetic construct
QVQLVQSGAEVKKPGASVKVSCKASGYTFTSYIIHWVRQAPGQGLEWIGYINPYNDGTKYNEKFKGRVTMTSDTSTSTVYMELSSLRSEDTAVYYCARGGIRAFMNYWGQGTLVTVSSASTKGPSVFPLAPSSKSTSGGTAALGCLVKDYFPEPVTVSWNSGALTSGVHTFPAVLQSSGLYSLSSVVTVPSSSLGTQTYICNVNHKPSNTKVDKKVEPKSCDKTHTCPPCPAPEAAGGPSVFLFPPKPKDTLMISRTPEVTCVVVDVSHEDPEVKFNWYVDGVEVHNAKTKPREEQYNSTYRVVSVLTVLHQDWLNGKEYKCKVSNKALPAPIEKTISKAKGQPREPQVCTLPPSRDELTKNQVSLSCAVKGFYPSDIAVEWESNGQPENNYKTTPPVLDSDGSFFLVSKLTVDKSRWQQGNVFSCSVMHEALHNRYTQKSLSLSPGK

SEQ ID NO: 3 - protein, 212 aa, synthetic construct
DIQMTQSPSSLSASVGDRVTITCKASQDVGTAVAWYQQKPGKAPKLLIYWASTRHTGVPSRFSGSGSGTDFTLTISSLQPEDFATYYCQHYISWTFGQGTKVEIKRTVAAPSVFIFPPSDEQLKSGTASVVCLLNNFYPREAKVQWKVDNALQSGNSQESVTEQDSKDSTYSLSSTLTLSKADYEKHKVYACEVTHQGLSSPVTKSFNRGEC

SEQ ID NO: 4 - protein, 227 aa, synthetic construct
DKTHTCPPCPAPEAAGGPSVFLFPPKPKDTLMISRTPEVTCVVVDVSHEDPEVKFNWYVDGVEVHNAKTKPREEQYNSTYRVVSVLTVLHQDWLNGKEYKCKVSNKALPAPIEKTISKAKGQPREPQVCTLPPSRDELTKNQVSLSCAVKGFYPSDIAVEWESNGQPENNYKTTPPVLDSDGSFFLVSKLTVDKSRWQQGNVFSCSVMHEALHNRYTQKSLSLSPGK

SEQ ID NO: 5 - protein, 448 aa, synthetic construct
QVQLVQSGAEVKKPGASVKVSCKASGYTFTSYIIHWVRQAPGQGLEWIGYINPYNDGTKYNEKFKGRVTMTSDTSTSTVYMELSSLRSEDTAVYYCARGGIRAFMNYWGQGTLVTVSSASTKGPSVFPLAPSSKSTSGGTAALGCLVKDYFPEPVTVSWNSGALTSGVHTFPAVLQSSGLYSLSSVVTVPSSSLGTQTYICNVNHKPSNTKVDKKVEPKSCDKTHTCPPCPAPELLGGPSVFLFPPKPKDTLMISRTPEVTCVVVDVSHEDPEVKFNWYVDGVEVHNAKTKPREEQYNSTYRVVSVLTVLHQDWLNGKEYKCKVSNKALPAPIEKTISKAKGQPREPQVYTLPPSRDELTKNQVSLTCLVKGFYPSDIAVEWESNGQPENNYKTTPPVLDSDGSFFLYSKLTVDKSRWQQGNVFSCSVMHEALHNHYTQKSLSLSPGK

SEQ ID NO: 6 - protein, 455 aa, synthetic construct
EVKLVESGGGLVQPGGSLKLSCAASGFTFNTYAMNWVRQAPGKGLEWVARIRSKYNNYATYYADSVKDRFTISRDDAKNTLYLQMNNLRTEDTAVYYCVRHGNFGNSYVSWFAYWGQGTLVTVSSASTKGPSVFPLAPSSKSTSGGTAALGCLVKDYFPEPVTVSWNSGALTSGVHTFPAVLQSSGLYSLSSVVTVPSSSLGTQTYICNVNHKPSNTKVDKKVEPKSCDKTHTCPPCPAPEAAGGPSVFLFPPKPKDTLMISRTPEVTCVVVDVSHEDPEVKFNWYVDGVEVHNAKTKPREEQYNSTYRVVSVLTVLHQDWLNGKEYKCKVSNKALPAPIEKTISKAKGQPREPQVYTLPPSRDELTKNQVSLTCLVKGFYPSDIAVEWESNGQPENNYKTTPPVLDSDGSFFLYSKLTVDKSRWQQGNVFSCSVMHEALHNHYTQKSLSLSPGK

SEQ ID NO: 7 - protein, 214 aa, synthetic construct
QAVVTQEPSLTVSPGGTVTLTCRSSTGAVTTSNYANWVQQKPGQAPRGLIGGTNKRAPGTPARFSGSLLGGKAALTLSGAQPEDEAEYYCALWYSNLWVFGGGTKLTVLGQPKANPTVTLFPPSSEELQANKATLVCLISDFYPGAVTVAWKADSSPVKAGVETTTPSKQSNNKYAASSYLSLTPEQWKSHRSYSCQVTHEGSTVEKTVAPTEC

SEQ ID NO: 8 - protein, 249 aa, synthetic construct
EVKLVESGGGLVQPGGSLKLSCAASGFTFNTYAMNWVRQAPGKGLEWVARIRSKYNNYATYYADSVKDRFTISRDDAKNTLYLQMNNLRTEDTAVYYCVRHGNFGNSYVSWFAYWGQGTLVTVSSGGGGSGGGGSGGGGSQAVVTQEPSLTVSPGGTVTLTCRSSTGAVTTSNYANWVQQKPGQAPRGLIGGTNKRAPGTPARFSGSLLGGKAALTLSGAQPEDEAEYYCALWYSNLWVFGGGTKLTVL

SEQ ID NO: 9 - protein, 118 aa, synthetic construct
QVQLVQSGAEVKKPGASVKVSCKASGYTFTSYIIHWVRQAPGQGLEWIGYINPYNDGTKYNEKFKGRVTMTSDTSTSTVYMELSSLRSEDTAVYYCARGGIRAFMNYWGQGTLVTVSS

SEQ ID NO: 10 - protein, 105 aa, synthetic construct
DIQMTQSPSSLSASVGDRVTITCKASQDVGTAVAWYQQKPGKAPKLLIYWASTRHTGVPSRFSGSGSGTDFTLTISSLQPEDFATYYCQHYISWTFGQGTKVEIK

SEQ ID NO: 11 - protein, 5 aa, synthetic construct
SYIIH

SEQ ID NO: 12 - protein, 17 aa, synthetic construct
YINPYNDGTKYNEKFKG

SEQ ID NO: 13 - protein, 9 aa, synthetic construct
GGIRAFMNY

SEQ ID NO: 14 - protein, 11 aa, synthetic construct
KASQDVGTAVA

SEQ ID NO: 15 - protein, 7 aa, synthetic construct
WASTRHT

SEQ ID NO: 16 - protein, 7 aa, synthetic construct
QHYISWT

SEQ ID NO: 17 - protein, 125 aa, synthetic construct
EVKLVESGGGLVQPGGSLKLSCAASGFTFNTYAMNWVRQAPGKGLEWVARIRSKYNNYATYYADSVKDRFTISRDDAKNTLYLQMNNLRTEDTAVYYCVRHGNFGNSYVSWFAYWGQGTLVTVSS

SEQ ID NO: 18 - protein, 109 aa, synthetic construct
QAVVTQEPSLTVSPGGTVTLTCRSSTGAVTTSNYANWVQQKPGQAPRGLIGGTNKRAPGTPARFSGSLLGGKAALTLSGAQPEDEAEYYCALWYSNLWVFGGGTKLTVL

SEQ ID NO: 19 - protein, 5 aa, synthetic construct
TYAMN

SEQ ID NO: 20 - protein, 19 aa, synthetic construct
RIRSKYNNYATYYADSVKD

SEQ ID NO: 21 - protein, 14 aa, synthetic construct
HGNFGNSYVSWFAY

SEQ ID NO: 22 - protein, 14 aa, synthetic construct
RSSTGAVTTSNYAN

SEQ ID NO: 23 - protein, 7 aa, synthetic construct
GTNKRAP

SEQ ID NO: 24 - protein, 9 aa, synthetic construct
ALWYSNLWV

SEQ ID NO: 25 - protein, 221 aa, synthetic construct
QVQLVQSGAEVKKPGASVKVSCKASGYTFTSYIIHWVRQAPGQGLEWIGYINPYNDGTKYNEKFKGRVTMTSDTSTSTVYMELSSLRSEDTAVYYCARGGIRAFMNYWGQGTLVTVSSASTKGPSVFPLAPSSKSTSGGTAALGCLVKDYFPEPVTVSWNSGALTSGVHTFPAVLQSSGLYSLSSVVTVPSSSLGTQTYICNVNHKPSNTKVDKKVEPKSC

SEQ ID NO: 26 - protein, 227 aa, synthetic construct
DKTHTCPPCPAPEAAGGPSVFLFPPKPKDTLMISRTPEVTCVVVDVSHEDPEVKFNWYVDGVEVHNAKTKPREEQYNSTYRVVSVLTVLHQDWLNGKEYKCKVSNKALPAPIEKTISKAKGQPREPQVYTLPPCRDELTKNQVSLWCLVKGFYPSDIAVEWESNGQPENNYKTTPPVLDSDGSFFLYSKLTVDKSRWQQGNVFSCSVMHEALHNHYTQKSLSLSPGK

SEQ ID NO: 27 - protein, 118 aa, synthetic construct
EVQLQQSGPELVKPGASVKMSCKASGYTFTSYIIHWVKQKPGQGLEWIGYINPYNDGTKYNEKFKGKATLTSDRSSSTAYMEVSSLTSEDSAVYYCARGGIRAFMNYWGQGTSVTVSS

SEQ ID NO: 28 - protein, 105 aa, synthetic construct
DIVMTQSHKFMSTSVGDRVSITCKASQDVGTAVAWYQQKPGQSPKLLIYWASTRHTGVPDRFTGSGSGTDFTLSISNVQSEDLADYFCQHYISWTFGGGTNLEIK